European Patent Specification EP 3 716 956 B1, published June 26, 2024. Title: ANTITUMOR TET2 MODULATING COMPOUNDS. Applicant: THE CLEVELAND CLINIC FOUNDATION. The sequence listing filed with the application follows.

SEQUENCE LISTING (3 sequences)

SEQ ID NO: 1 - protein, 318 aa, Homo sapiens
EDNLQSLATRLAPIYKQYAPVAYQNQVEYENVARECRLGSKEGRPFSGVTACLDFCAHPHRDIHNMNNGSTVVCTLTREDNRSLGVIPQDEQLHVLPLYKLSDTDEFGSKEGMEAKIKSGPNHQPSFLTSPQDLASSPMEEDEQHSEADEPPSDEPLSDDPLSPAEEKLPHIDEYWSDSEHIFLDANIGGVAIAPAHGSVLIECARRELHATTPVEHPNRNHPTRLSLVFYQHKNLNKPQHGFELNKIKFEAKEAKNKKMKASEQKDQAANEGPEQSSEVNELNQIPSHKALTLTHDNVVTVSPYALTHVAGPYNHWV

SEQ ID NO: 2 - protein, 368 aa, Homo sapiens
ESHLQNLSTLMAPTYKKLAPDAYNNQIEYEHRAPECRLGLKEGRPFSGVTACLDFCAHAHRDLHNMQNGSTLVCTLTREDNREFGGKPEDEQLHVLPLYKVSDVDEFGSVEAQEEKKRSGEHHSPSHIIHNVSAAPGMFNSSLHALHLQNKENDMLSHTANGLSKMLPALNHDRTACVQGGLHKLSDANGQEKQPLALVQGVASGAEDNDEVWSDSEQSFLDPDIGGVAVAPTHGSILIECAKRELHATTPLKNPNRNHPTRISLVFYQHKSMNEPKHGLALWEAKMAEKAREKEEECEKYGPDYVPQKSHGKKVKREPAEPHETSEPTYLRFIKSLAERTMSVTTDSTVTTSPYAFTRVTGPYNRYI

SEQ ID NO: 3 - protein, 392 aa, Homo sapiens
RKSFQDLATEVAPLYKRLAPQAYQNQVTNEEIAIDCRLGLKEGRPFAGVTACMDFCAHAHKDQHNLYNGCTVVCTLTKEDNRCVGKIPEDEQLHVLPLYKMANTDEFGSEENQNAKVGSGALAGPSLTEKPWALGAGDFNSALKGSPGFQDKLWNPMKGEEGRIPAAGASQLDRAWQSFGLPLGSSEKLFGALKSEEKLWDPFSLEEGPAEEPPSKGAVKEEKGGGGAEEEEEELWSDSEHNFLDENIGGVAVAPAHGSILIECARRELHATTPLKKPNRCHPTRISLVFYQHKNLNQPNHGLALWEAKMKQLAERARARQEEAARLGLGQQEAKLYGKKRKWGGTVVAEPQQKEKKGVVPTRQALAVPTDSAVTVSSYAYTKVTGPYSRWI